European Patent Specification EP 3 664 831 B1, published June 14, 2023. Title: ANTI-NEURODEGENERATIVE THERAPEUTIC, METHOD OF MANUFACTURE, AND USE. Applicant: University of Kentucky Research Foundation BRADLEY, Luke H. GASH, Don M. GERHARDT, Greg A. The sequence listing filed with the application follows.

SEQUENCE LISTING (11 sequences)

SEQ ID NO: 1 - protein, 6 aa, Artificial Sequence
  SYNTHESIZED
  MISC_FEATURE (6)..(6): AMIDATION
LAPAED

SEQ ID NO: 2 - protein, 6 aa, Artificial Sequence
  SYNTHESIZED
  MISC_FEATURE (6)..(6): AMIDATION
EAPFED

SEQ ID NO: 3 - protein, 6 aa, Artificial Sequence
  SYNTHESIZED
  MISC_FEATURE (6)..(6): AMIDATION
LAPYED

SEQ ID NO: 4 - protein, 6 aa, Artificial Sequence
  SYNTHESIZED
  MISC_FEATURE (6)..(6): AMIDATION can either be present or absent
LGPFSE

SEQ ID NO: 5 - protein, 8 aa, Artificial Sequence
  SYNTHESIZED
CLGPFSEC

SEQ ID NO: 6 - protein, 5 aa, Artificial Sequence
  SYNTHESIZED
  MISC_FEATURE (2)..(2): Xaa is D-Ala
  MISC_FEATURE (4)..(4): Xaa is D-Lys
  MISC_FEATURE (5)..(5): AMIDATION
WXPXD

SEQ ID NO: 7 - protein, 6 aa, Artificial Sequence
  SYNTHESIZED
  MISC_FEATURE (1)..(1): Xaa is D-Glu
  MISC_FEATURE (5)..(5): Xaa is D-Ala
  MISC_FEATURE (6)..(6): AMIDATION
XAPFXG

SEQ ID NO: 8 - protein, 5 aa, Artificial Sequence
  SYNTHESIZED
  MISC_FEATURE (2)..(2): Xaa is deuterated Lys
  MISC_FEATURE (4)..(4): Xaa is D-Phe
  MISC_FEATURE (5)..(5): Xaa is deuterated Leu
  MISC_FEATURE (5)..(5): AMIDATION
EXPXX

SEQ ID NO: 9 - protein, 6 aa, Artificial Sequence
  SYNTHESIZED
  MISC_FEATURE (1)..(1): Xaa is acylated-Leu
  MISC_FEATURE (2)..(2): Xaa is D-Met
  MISC_FEATURE (5)..(5): Xaa is deuterated Ser
XXPAXF

SEQ ID NO: 10 - protein, 5 aa, Artificial Sequence
  SYNTHESIZED
  MISC_FEATURE (5)..(5): AMIDATION
EAPAE

SEQ ID NO: 11 - protein, 6 aa, Artificial Sequence
  SYNTHESIZED
  MISC_FEATURE (6)..(6): AMIDATION
EAPAED